European Patent Specification EP 3 838 923 B1, published May 1, 2024. Title: ANTIBODIES AND VACCINES FOR USE IN TREATING ROR1 CANCERS AND INHIBITING METASTASIS. Applicant: THE REGENTS OF THE UNIVERSITY OF CALIFORNIA. The sequence listing filed with the application follows.

SEQUENCE LISTING (46 sequences)

SEQ ID NO: 1 - protein, 116 aa, Artificial mouse
  Synthetic construct
EIQLQQSGPVLVKPGASVKVSCKASGYAFTAYNIHWVRQSHGKRLEWIGSFDPYDGGSSYNQKFKDKATLTVDKSSTTAYMHLNSLTSEDSAVYYCARGWYYFDYWGHGTTLTVSS

SEQ ID NO: 2 - DNA, 348 bp, Mus musculus
gagatccagctgcagcagtctggacctgtcctggtgaagcctggggcttcagtgaaggtttcttgcaaggcttctggttatgcattcactgcctacaacatacactgggtgagacagagccatggaaagcgccttgagtggattggatcttttgatccttacgatggtggtagtagttacaaccagaagttcaaggacaaagccacattgactgtagacaaatcttccaccacagcctacatgcatctcaacagcctgacatctgaggactctgcagtctattactgtgcaagggggtggtactactttgactactggggccacgggaccactctcacagtctcctca

SEQ ID NO: 3 - protein, 108 aa, Mus musculus
DVQITQSPSYLAASPGETITINCRASKSISKYLAWYQEKPGKTNKLLIYSGSTLQSGIPSRFRGSGSGTDFTLTISSLEPEDFAMYYCQQHDESPYTFGEGTKLEIKR

SEQ ID NO: 4 - DNA, 324 bp, Mus musculus
gacgtccagataacccagtctccatcttatcttgctgcatctcctggagaaaccattactattaattgcagggcaagtaagagcattagcaaatatttagcctggtatcaagagaaacctgggaaaactaataagctccttatctactctggatccactttgcaatctggaattccatcaagattcaggggcagtggatctggtacagatttcactctcaccatcagtagcctggagcctgaagattttgcaatgtattactgtcaacagcatgatgaatccccgtacacgttcggagaggggaccaagctggaaataaaacgg

SEQ ID NO: 5 - protein, 116 aa, Artificial Sequence
  Synthetic construct
QVQLQESGPGLVKPSQTLSLTCTVSGYAFTAYNIHWVRQAPGQGLEWMGSFDPYDGGSSYNQKFKDRLTISKDTSKNQVVLTMTNMDPVDTATYYCARGWYYFDYWGHGTLVTVSS

SEQ ID NO: 6 - DNA, 348 bp, Artificial Sequence
  Synthetic construct
caggtgcagctgcaggagtcgggcccaggactggtgaagccttcacagaccctgtccctcacctgcactgtctctggttatgcattcactgcctacaacatacactgggtgcgacaggcccctggacaagggcttgagtggatgggttcttttgatccttacgatggtggtagtagttacaaccagaagttcaaggacagactcaccatctccaaggacacctccaaaaaccaggtggtccttacaatgaccaacatggaccctgtggacacagccacgtattactgtgcaagagggtggtactactttgactactggggccacggaaccctggtcaccgtctcctca

SEQ ID NO: 7 - protein, 107 aa, Artificial Sequence
  Synthetic construct
DIVMTQTPLSLPVTPGEPASISCRASKSISKYLAWYQQKPGQAPRLLIYSGSTLQSGIPPRFSGSGYGTDFTLTINNIESEDAAYYFCQQHDESPYTFGEGTKVEIK

SEQ ID NO: 8 - DNA, 321 bp, Artificial Sequence
  Synthetic construct
gatattgtgatgacccagactccactctccctgcccgtcacccctggagagccggcctccatctcctgcagggcaagtaagagcattagcaaatatttagcctggtaccagcagaaacctggccaggctcccaggctcctcatctattctggatccactttgcaatctgggatcccacctcgattcagtggcagcgggtatggaacagattttaccctcacaattaataacatagaatctgaggatgctgcatattacttctgtcaacagcatgatgaatccccgtacacgttcggcgaggggaccaaggtggaaatcaaa

SEQ ID NO: 9 - protein, 116 aa, Artificial Sequence; identical to SEQ ID NO: 5
  Synthetic construct

SEQ ID NO: 10 - DNA, 348 bp, Artificial Sequence; identical to SEQ ID NO: 6
  Synthetic construct

SEQ ID NO: 11 - protein, 107 aa, Artificial Sequence
  Synthetic construct
DVVMTQSPLSLPVTLGQPASISCRASKSISKYLAWYQQKPGKAPKLLIYSGSTLQSGIPPRFSGSGYGTDFTLTINNIESEDAAYYFCQQHDESPYTFGEGTKVEIK

SEQ ID NO: 12 - DNA, 321 bp, Artificial Sequence
  Synthetic construct
gatgttgtgatgactcagtctccactctccctgcccgtcacccttggacagccggcctccatctcctgcagggcaagtaagagcattagcaaatatttagcctggtatcagcagaaaccagggaaagctcctaagctcctgatctattctggatccactttgcaatctgggatcccacctcgattcagtggcagcgggtatggaacagattttaccctcacaattaataacatagaatctgaggatgctgcatattacttctgtcaacagcatgatgaatccccgtacacgttcggcgaggggaccaaggtggaaatcaaa

SEQ ID NO: 13 - protein, 116 aa, Artificial Sequence
  Synthetic construct
QVQLQESGPGLVKPSQTLSLTCTVSGYAFTAYNIHWIRQPPGKGLEWIGSFDPYDGGSSYNQKFKDRLTISKDTSKNQVVLTMTNMDPVDTATYYCARGWYYFDYWGHGTLVTVSS

SEQ ID NO: 14 - DNA, 348 bp, Artificial Sequence
  Synthetic construct
caggtgcagctgcaggagtcgggcccaggactggtgaagccttcacagaccctgtccctcacctgcactgtctctggttatgcattcactgcctacaacatacactggatccgccagcccccagggaaggggctggagtggattggttcttttgatccttacgatggtggtagtagttacaaccagaagttcaaggacagactcaccatctccaaggacacctccaaaaaccaggtggtccttacaatgaccaacatggaccctgtggacacagccacgtattactgtgcaagagggtggtactactttgactactggggccacggaaccctggtcaccgtctcctca

SEQ ID NO: 15 - protein, 107 aa, Artificial Sequence; identical to SEQ ID NO: 7
  Synthetic construct

SEQ ID NO: 16 - DNA, 321 bp, Artificial Sequence; identical to SEQ ID NO: 8
  Synthetic construct

SEQ ID NO: 17 - protein, 116 aa, Artificial Sequence; identical to SEQ ID NO: 13
  Synthetic construct

SEQ ID NO: 18 - DNA, 348 bp, Artificial Sequence; identical to SEQ ID NO: 14
  Synthetic construct

SEQ ID NO: 19 - protein, 107 aa, Artificial Sequence; identical to SEQ ID NO: 11
  Synthetic construct

SEQ ID NO: 20 - DNA, 321 bp, Artificial Sequence; identical to SEQ ID NO: 12
  Synthetic construct

SEQ ID NO: 21 - protein, 252 aa, Artificial Sequence
  Synthetic construct
DIVMTTQTPLSLPVTPGEPASISCRASKSISKYLAWYQQKPGQAPRLLIYSGSTLQSGIPPRFSGSGYGTDFTLTINNIESEDAAYYFCQQHDESPYTFGEGTKVEIKGGGGSGSTSGSGKPGSGEGSTKGGGGGSQVQLQESGPGLVKPSQTLSLTCTVSGYAFTAYNIHWVRQAPGQGLEWMGSFDPYDGGSSYNQKFKDRLTISKDTSKNQVVLTMTNMDPVDTATYYCARGWYYFDYWGHGTLVTVSS

SEQ ID NO: 22 - DNA, 753 bp, Artificial Sequence
  Synthetic construct
gatattgtgatgacccagactccactctccctgcccgtcacccctggagagccggcctccatctcctgcagggcaagtaagagcattagcaaatatttagcctggtaccagcagaaacctggccaggctcccaggctcctcatctattctggatccactttgcaatctgggatcccacctcgattcagtggcagcgggtatggaacagattttaccctcacaattaataacatagaatctgaggatgctgcatattacttctgtcaacagcatgatgaatccccgtacacgttcggcgaggggaccaaggtggaaatcaaaggtggtggtggtagcggctccacctctggatccggcaagcccggatctggcgagggatccaccaagggcggaggaggaggaagtcaggtgcagctgcaggagtcgggcccaggactggtgaagccttcacagaccctgtccctcacctgcactgtctctggttatgcattcactgcctacaacatacactgggtgcgacaggcccctggacaagggcttgagtggatgggttcttttgatccttacgatggtggtagtagttacaaccagaagttcaaggacagactcaccatctccaaggacacctccaaaaaccaggtggtccttacaatgaccaacatggaccctgtggacacagccacgtattactgtgcaagagggtggtactactttgactactggggccacggaaccctggtcaccgtctcctca

SEQ ID NO: 23 - protein, 251 aa, Artificial Sequence
  Synthetic construct
DVVMTQSPLSLPVTLGQPASISCRASKSISKYLAWYQQKPGKAPKLLIYSGSTLQSGIPPRFSGSGYGTDFTLTINNIESEDAAYYFCQQHDESPYTFGEGTKVEIKGGGGSGSTSGSGKPGSGEGSTKGGGGGSQVQLQESGPGLVKPSQTLSLTCTVSGYAFTAYNIHWVRQAPGQGLEWMGSFDPYDGGSSYNQKFKDRLTISKDTSKNQVVLTMTNTDPVDTATYYCARGWYYFDYWGHGTLVTVSS

SEQ ID NO: 24 - DNA, 753 bp, Artificial Sequence
  Synthetic construct
gatgttgtgatgactcagtctccactctccctgcccgtcacccttggacagccggcctccatctcctgcagggcaagtaagagcattagcaaatatttagcctggtatcagcagaaaccagggaaagctcctaagctcctgatctattctggatccactttgcaatctgggatcccacctcgattcagtggcagcgggtatggaacagattttaccctcacaattaataacatagaatctgaggatgctgcatattacttctgtcaacagcatgatgaatccccgtacacgttcggcgaggggaccaaggtggaaatcaaaggtggtggtggtagcggctccacctctggatccggcaagcccggatctggcgagggatccaccaagggcggaggaggaggaagtcaggtgcagctgcaggagtcgggcccaggactggtgaagccttcacagaccctgtccctcacctgcactgtctctggttatgcattcactgcctacaacatacactgggtgcgacaggcccctggacaagggcttgagtggatgggttcttttgatccttacgatggtggtagtagttacaaccagaagttcaaggacagactcaccatctccaaggacacctccaaaaaccaggtggtccttacaatgaccaacatggaccctgtggacacagccacgtattactgtgcaagagggtggtactactttgactactggggccacggaaccctggtcaccgtctcctca

SEQ ID NO: 25 - protein, 22 aa, Artificial Sequence
  Synthetic construct
VATNGKEVVSSTGVLFVKFGPC

SEQ ID NO: 26 - protein, 16 aa, Artificial Sequence
  Synthetic construct
EVVSSTGVLFVKFGPC

SEQ ID NO: 27 - protein, 8 aa, Artificial Sequence
  Synthetic construct
GYAFTAYN

SEQ ID NO: 28 - protein, 8 aa, Artificial Sequence
  Synthetic construct
FDPYDGGS

SEQ ID NO: 29 - protein, 7 aa, Artificial Sequence
  Synthetic construct
GWYYFDY

SEQ ID NO: 30 - protein, 6 aa, Artificial Sequence
  Synthetic construct
KSISKY

SEQ ID NO: 31 - protein, 3 aa, Artificial Sequence
  Synthetic construct
SGS

SEQ ID NO: 32 - protein, 8 aa, Artificial Sequence
  Synthetic construct
QQHDESPY

SEQ ID NO: 33 - protein, 15 aa, Artificial Sequence
  Synthetic construct
SGYAFTAYNIHWVRQ

SEQ ID NO: 34 - protein, 18 aa, Artificial Sequence
  Synthetic construct
GSFDPYDGGSSYNQKFKD

SEQ ID NO: 35 - protein, 23 aa, Artificial Sequence
  Synthetic construct
YYCARGWYYFDYWGHGTLVTVSS

SEQ ID NO: 36 - protein, 14 aa, Artificial Sequence
  Synthetic construct
CRASKSISKYLAWY

SEQ ID NO: 37 - protein, 12 aa, Artificial Sequence
  Synthetic construct
LLIYSGSTLQSG

SEQ ID NO: 38 - protein, 20 aa, Artificial Sequence
  Synthetic construct
CQQHDESPYTFGEGTKVEIK

SEQ ID NO: 39 - protein, 117 aa, Mus musculus
QVQLKESGPGLVAPSQTLSITCTVSGFSLTSYGVHWVRQPPGKGLEWLGVIWAGGFTNYNSALKSRLSISKDNSKSQVLLKMTSLQTDDTAMYYCARRGSSYSMDYWGQGTSVTVSS

SEQ ID NO: 40 - DNA, 351 bp, Mus musculus
caggtgcagctgaaggagtcaggacctggcctggtggcgccctcacagactctgtccatcacttgcactgtctctgggttttcattaaccagttatggtgtacactgggttcgccagcctccaggaaagggtctggagtggctgggagtaatatgggctggtggattcacaaattataattcggctctcaagtccagactgagcatcagcaaagacaactccaagagccaagttctcttaaaaatgaccagtctgcaaactgatgacacagccatgtactactgtgccaggagaggtagttcctattctatggactattggggtcaaggaacctcagtcaccgtctcctca

SEQ ID NO: 41 - protein, 106 aa, Mus musculus
EIVLSQSPAITAASLGQKVTITCSASSNVSYIHWYQQRSGTSPRPWIYEISKLASGVPVRFSGSGSGTSYSLTISSMEAEDAAIYYCQQWNYPLITFGSGTKLEIQ

SEQ ID NO: 42 - DNA, 318 bp, Mus musculus
gaaattgtgctctctcagtctccagccatcacagctgcatctctgggccaaaaggtcaccatcacctgcagtgccagttcaaatgtaagttacatccactggtaccagcagaggtcaggcacctcccccagaccatggatttatgaaatatccaaactggcttctggagtcccagttcgcttcagtggcagtgggtctgggacctcttactctctcacaatcagcagcatggaggctgaagatgctgccatttattattgtcagcagtggaattatcctcttatcacgttcggctcggggacaaagttggaaatacaa

SEQ ID NO: 43 - protein, 119 aa, Mus musculus
EVKLVESGGGLVKPGGSLKLSCAASGFTFSSYAMSWVRQIPEKRLEWVASISRGGTTYYPDSVKGRFTISRDNVRNILYLQMSSLRSEDTAMYYCGRYDYDGYYAMDYWGQGTSVTVSS

SEQ ID NO: 44 - DNA, 357 bp, Mus musculus
gaagtgaaactggtggagtctgggggaggcttagtgaagcctggagggtccctgaaactctcctgtgcagcctctggattcactttcagtagctatgccatgtcttgggttcgccagattccagagaagaggctggagtgggtcgcatccattagtcgtggtggtaccacctactatccagacagtgtgaagggccgattcaccatctccagagataatgtcaggaacatcctgtacctgcaaatgagcagtctgaggtctgaggacacggccatgtattactgtggaagatatgattacgacgggtactatgcaatggactactggggtcaaggaacctcagtcaccgtctcctca

SEQ ID NO: 45 - protein, 107 aa, Mus musculus
DIKMTQSPSSMYASLGERVTITCKASPDINSYLSWFQQKPGKSPKTLIYRANRLVDGVPSRFSGGGSGQDYSLTINSLEYEDMGIYYCLQYDEFPYTFGGGTKLEMK

SEQ ID NO: 46 - DNA, 322 bp, Mus musculus
gacatcaagatgacccagtctccatcttccatgtatgcatctctaggagagagagtcactatcacttgcaaggcgagtccggacattaatagctatttaagctggttccagcagaaaccagggaaatctcctaagaccctgatctatcgtgcaaacagattggttgatggggtcccatcaaggttcagtggcggtggatctgggcaagattattctctcaccatcaacagcctggagtatgaagatatgggaatttattattgtctacagtatgatgaatttccgtacacgttcggaggggggaccaagctggaaatgaaac